European Patent Application EP 4 789 684 A1, published August 12, 2026. Title: ANTI-ENDOGLIN ANTIBODY-DRUG CONJUGATES. Applicant: Oncomatryx Biopharma, S.L. The sequence listing filed with the application follows.

SEQUENCE LISTING (26 sequences)

SEQ ID NO: 1 - protein, 467 aa, synthetic construct
  REGION 1..467: note = Synthetic sequence: Anti-human Endoglin A5-IgG1-HC
METDTLLLWVLLLWVPGSTGEVQLLESGGGLVQPGGSLRLSCAASGFTFSSYAMSWVRQAPGKGLEWVSAIYGSDGDTTYADSVKGRFTISRDNSKNTLYLQMNSLRAEDTAVYYCARVFYTAGFDYWGQGTLVTVSSASTKGPSVFPLAPSSKSTSGGTAALGCLVKDYFPEPVTVSWNSGALTSGVHTFPAVLQSSGLYSLSSVVTVPSSSLGTQTYICNVNHKPSNTKVDKKVEPKSCDKTHTCPPCPAPPVAGPSVFLFPPKPKDTLMISRTPEVTCVVVDVSHEDPEVKFNWYVDGVEVHNAKTKPREEQYNSTYRVVSVLTVLHQDWLNGKEYKCKVSNKGLPSSIEKTISKAKGQPREPQVYTLPPSRDELTKNQVSLTCLVKGFYPSDIAVEWESNGQPENNYKTTPPVLDSDGSFFLYSKLTVDKSRWQQGNVFSCSVMHEALHNHYTQKSLSLSPGK

SEQ ID NO: 2 - protein, 234 aa, synthetic construct
  REGION 1..234: note = Synthetic sequence: Anti-human Endoglin A5-IgG1-LC
METDTLLLWVLLLWVPGSTGDIELTQSPSSLSASVGDRVTITCRASQSISSSLNWYQQKPGKAPKLLIYAASSLQSGVPSRFSGSGSGTDFTLTISSLQPEDFATYYCQQAPAKPPTFGQGTKLEIKRTVAAPSVFIFPPSDEQLKSGTASVVCLLNNFYPREAKVQWKVDNALQSGNSQESVTEQDSKDSTYSLSSTLTLSKADYEKHKVYACEVTHQGLSSPVTKSFNRGEC

SEQ ID NO: 3 - protein, 447 aa, synthetic construct
  REGION 1..447: note = Synthetic sequence: A5-IgG1-HC - without signal sequence
EVQLLESGGGLVQPGGSLRLSCAASGFTFSSYAMSWVRQAPGKGLEWVSAIYGSDGDTTYADSVKGRFTISRDNSKNTLYLQMNSLRAEDTAVYYCARVFYTAGFDYWGQGTLVTVSSASTKGPSVFPLAPSSKSTSGGTAALGCLVKDYFPEPVTVSWNSGALTSGVHTFPAVLQSSGLYSLSSVVTVPSSSLGTQTYICNVNHKPSNTKVDKKVEPKSCDKTHTCPPCPAPPVAGPSVFLFPPKPKDTLMISRTPEVTCVVVDVSHEDPEVKFNWYVDGVEVHNAKTKPREEQYNSTYRVVSVLTVLHQDWLNGKEYKCKVSNKGLPSSIEKTISKAKGQPREPQVYTLPPSRDELTKNQVSLTCLVKGFYPSDIAVEWESNGQPENNYKTTPPVLDSDGSFFLYSKLTVDKSRWQQGNVFSCSVMHEALHNHYTQKSLSLSPGK

SEQ ID NO: 4 - protein, 214 aa, synthetic construct
  REGION 1..214: note = Synthetic sequence: A5-IgG1-LC - without signal sequence
DIELTQSPSSLSASVGDRVTITCRASQSISSSLNWYQQKPGKAPKLLIYAASSLQSGVPSRFSGSGSGTDFTLTISSLQPEDFATYYCQQAPAKPPTFGQGTKLEIKRTVAAPSVFIFPPSDEQLKSGTASVVCLLNNFYPREAKVQWKVDNALQSGNSQESVTEQDSKDSTYSLSSTLTLSKADYEKHKVYACEVTHQGLSSPVTKSFNRGEC

SEQ ID NO: 5 - protein, 118 aa, synthetic construct
  REGION 1..118: note = Synthetic sequence: A5-VH
EVQLLESGGGLVQPGGSLRLSCAASGFTFSSYAMSWVRQAPGKGLEWVSAIYGSDGDTTYADSVKGRFTISRDNSKNTLYLQMNSLRAEDTAVYYCARVFYTAGFDYWGQGTLVTVSS

SEQ ID NO: 6 - protein, 108 aa, synthetic construct
  REGION 1..108: note = Synthetic sequence: A5-VL
DIELTQSPSSLSASVGDRVTITCRASQSISSSLNWYQQKPGKAPKLLIYAASSLQSGVPSRFSGSGSGTDFTLTISSLQPEDFATYYCQQAPAKPPTFGQGTKLEIKR

SEQ ID NO: 7 - protein, 5 aa, synthetic construct
  REGION 1..5: note = Synthetic sequence: A5-CDRH1
SYAMS

SEQ ID NO: 8 - protein, 11 aa, synthetic construct
  REGION 1..11: note = Synthetic sequence: A5-CDRH2
AIYGSDGDTTY

SEQ ID NO: 9 - protein, 9 aa, synthetic construct
  REGION 1..9: note = Synthetic sequence: A5-CDRH3
VFYTAGFDY

SEQ ID NO: 10 - protein, 11 aa, synthetic construct
  REGION 1..11: note = Synthetic sequence: A5-CDRL1
RASQSISSSLN

SEQ ID NO: 11 - protein, 7 aa, synthetic construct
  REGION 1..7: note = Synthetic sequence: A5-CDRL2
AASSLQS

SEQ ID NO: 12 - protein, 9 aa, synthetic construct
  REGION 1..9: note = Synthetic sequence: A5-CDRL3
QQAPAKPPT

SEQ ID NO: 13 - protein, 466 aa, synthetic construct
  REGION 1..466: note = Synthetic sequence: Anti-murine Endoglin mE12-IgG1-HC
METDTLLLWVLLLWVPGSTGEVQLVESGGGVVQPGRSLRLSCAASGFTFSSYGMHWVRQAPGKGLVWVSRINSDGSSTSYADSVKGRFTISRDNSKNTLYLQMNSLRAEDTAVYYCARATGTWVMSWGQGTLVTVSSASTKGPSVFPLAPSSKSTSGGTAALGCLVKDYFPEPVTVSWNSGALTSGVHTFPAVLQSSGLYSLSSVVTVPSSSLGTQTYICNVNHKPSNTKVDKKVEPKSCDKTHTCPPCPAPPVAGPSVFLFPPKPKDTLMISRTPEVTCVVVDVSHEDPEVKFNWYVDGVEVHNAKTKPREEQYNSTYRVVSVLTVLHQDWLNGKEYKCKVSNKGLPSSIEKTISKAKGQPREPQVYTLPPSRDELTKNQVSLTCLVKGFYPSDIAVEWESNGQPENNYKTTPPVLDSDGSFFLYSKLTVDKSRWQQGNVFSCSVMHEALHNHYTQKSLSLSPGK

SEQ ID NO: 14 - protein, 232 aa, synthetic construct
  REGION 1..232: note = Synthetic sequence: Anti-murine Endoglin mE12-IgG1-LC
METDTLLLWVLLLWVPGSTGSSELIQDPAVSVALGQTVRITCQGDSLRSYYASWYQQKPGQAPVLVIYGKNNRPSGIPDRFSGSSSGNTASLTITGAQAEDEADYYCNSRDSSGTVFGGGTKLTVLGQPKANPTVTLFPPSSEELQANKATLVCLISDFYPGAVTVAWKADGSPVKAGVETTKPSKQSNNKYAASSYLSLTPEQWKSHRSYSCQVTHEGSTVEKTVAPTECS

SEQ ID NO: 15 - protein, 446 aa, synthetic construct
  REGION 1..446: note = Synthetic sequence: mE12-IgG1-HC - without signal sequence
EVQLVESGGGVVQPGRSLRLSCAASGFTFSSYGMHWVRQAPGKGLVWVSRINSDGSSTSYADSVKGRFTISRDNSKNTLYLQMNSLRAEDTAVYYCARATGTWVMSWGQGTLVTVSSASTKGPSVFPLAPSSKSTSGGTAALGCLVKDYFPEPVTVSWNSGALTSGVHTFPAVLQSSGLYSLSSVVTVPSSSLGTQTYICNVNHKPSNTKVDKKVEPKSCDKTHTCPPCPAPPVAGPSVFLFPPKPKDTLMISRTPEVTCVVVDVSHEDPEVKFNWYVDGVEVHNAKTKPREEQYNSTYRVVSVLTVLHQDWLNGKEYKCKVSNKGLPSSIEKTISKAKGQPREPQVYTLPPSRDELTKNQVSLTCLVKGFYPSDIAVEWESNGQPENNYKTTPPVLDSDGSFFLYSKLTVDKSRWQQGNVFSCSVMHEALHNHYTQKSLSLSPGK

SEQ ID NO: 16 - protein, 212 aa, synthetic construct
  REGION 1..212: note = Synthetic sequence: mE12-IgG1-LC - without signal sequence
SSELIQDPAVSVALGQTVRITCQGDSLRSYYASWYQQKPGQAPVLVIYGKNNRPSGIPDRFSGSSSGNTASLTITGAQAEDEADYYCNSRDSSGTVFGGGTKLTVLGQPKANPTVTLFPPSSEELQANKATLVCLISDFYPGAVTVAWKADGSPVKAGVETTKPSKQSNNKYAASSYLSLTPEQWKSHRSYSCQVTHEGSTVEKTVAPTECS

SEQ ID NO: 17 - protein, 117 aa, synthetic construct
  REGION 1..117: note = Synthetic sequence: mE12-VH
EVQLVESGGGVVQPGRSLRLSCAASGFTFSSYGMHWVRQAPGKGLVWVSRINSDGSSTSYADSVKGRFTISRDNSKNTLYLQMNSLRAEDTAVYYCARATGTWVMSWGQGTLVTVSS

SEQ ID NO: 18 - protein, 107 aa, synthetic construct
  REGION 1..107: note = Synthetic sequence: mE12-VL
SSELIQDPAVSVALGQTVRITCQGDSLRSYYASWYQQKPGQAPVLVIYGKNNRPSGIPDRFSGSSSGNTASLTITGAQAEDEADYYCNSRDSSGTVFGGGTKLTVLG

SEQ ID NO: 19 - protein, 5 aa, synthetic construct
  REGION 1..5: note = Synthetic sequence: mE12-CDRH1
SYGMH

SEQ ID NO: 20 - protein, 17 aa, synthetic construct
  REGION 1..17: note = Synthetic sequence: mE12-CDRH2
RINSDGSSTSYADSVKG

SEQ ID NO: 21 - protein, 8 aa, synthetic construct
  REGION 1..8: note = Synthetic sequence: mE12-CDRH3
ATGTWVMS

SEQ ID NO: 22 - protein, 11 aa, synthetic construct
  REGION 1..11: note = Synthetic sequence: mE12-CDRL1
QGDSLRSYYAS

SEQ ID NO: 23 - protein, 7 aa, synthetic construct
  REGION 1..7: note = Synthetic sequence: mE12-CDRL2
GKNNRPS

SEQ ID NO: 24 - protein, 9 aa, synthetic construct
  REGION 1..9: note = Synthetic sequence: mE12-CDRL3
NSRDSSGTV

SEQ ID NO: 25 - protein, 656 aa, Homo sapiens
MDRGTLPLAVALLLASCSLSPTSLAETVHCDLQPVGPERGEVTYTTSQVSKGCVAQAPNAILEVHVLFLEFPTGPSQLELTLQASKQNGTWPREVLLVLSVNSSVFLHLQALGIPLHLAYNSSLVTFQEPPGVNTTELPSFPKTQILEWAAERGPITSAAELNDPQSILLRLGQAQGSLSFCMLEASQDMGRTLEWRPRTPALVRGCHLEGVAGHKEAHILRVLPGHSAGPRTVTVKVELSCAPGDLDAVLILQGPPYVSWLIDANHNMQIWTTGEYSFKIFPEKNIRGFKLPDTPQGLLGEARMLNASIVASFVELPLASIVSLHASSCGGRLQTSPAPIQTTPPKDTCSPELLMSLIQTKCADDAMTLVLKKELVAHLKCTITGLTFWDPSCEAEDRGDKFVLRSAYSSCGMQVSASMISNEAVVNILSSSSPQRKKVHCLNMDSLSFQLGLYLSPHFLQASNTIEPGQQSFVQVRVSPSVSEFLLQLDSCHLDLGPEGGTVELIQGRAAKGNCVSLLSPSPEGDPRFSFLLHFYTVPIPKTGTLSCTVALRPKTGSQDQEVHRTVFMRLNIISPDLSGCTSKGLVLPAVLGITFGAFLIGALLTAALWYIYSHTRSPSKREPVVAVAAPASSESSSTNHSIGSTQSTPCSTSS

SEQ ID NO: 26 - protein, 653 aa, Mus musculus
MDRGVLPLPITLLFVIYSFVPTTGLAERVGCDLQPVDPTRGEVTFTTSQVSEGCVAQAANAVREVHVLFLDFPGMLSHLELTLQASKQNGTETQEVFLVLVSNKNVFVKFQAPEIPLHLAYDSSLVIFQGQPRVNITVLPSLTSRKQILDWAATKGAITSIAALDDPQSIVLQLGQDPKAPFLCLPEAHKDMGATLEWQPRAQTPVQSCRLEGVSGHKEAYILRILPGSEAGPRTVTVMMELSCTSGDAILILHGPPYVSWFIDINHSMQILTTGEYSVKIFPGSKVKGVELPDTPQGLIAEARKLNASIVTSFVELPLVSNVSLRASSCGGVFQTTPAPVVTTPPKDTCSPVLLMSLIQPKCGNQVMTLALNKKHVQTLQCTITGLTFWDSSCQAEDTDDHLVLSSAYSSCGMKVTAHVVSNEVIISFPSGSPPLRKKVQCIDMDSLSFQLGLYLSPHFLQASNTIELGQQAFVQVSVSPLTSEVTVQLDSCHLDLGPEGDMVELIQSRTAKGSCVTLLSPSPEGDPRFSFLLRVYMVPTPTAGTLSCNLALRPSTLSQEVYKTVSMRLNIVSPDLSGKGLVLPSVLGITFGAFLIGALLTAALWYIYSHTRGPSKREPVVAVAAPASSESSSTNHSIGSTQSTPCSTSSMA